European Patent Specification EP 3 864 039 B1, published December 6, 2023. Title: NEUROENDOCRINE CANCER TARGETED THERAPY. Applicant: The UAB Research Foundation. The sequence listing filed with the application follows.

SEQUENCE LISTING (30 sequences)

SEQ ID NO: 1 - protein, 5 aa, Artificial Sequence
  Synthetic Construct
DYHLN

SEQ ID NO: 2 - protein, 18 aa, Artificial Sequence
  Synthetic Construct
IRNKRYGYRTEYSASVKG

SEQ ID NO: 3 - protein, 8 aa, Artificial Sequence
  Synthetic Construct
DFYDPFAY

SEQ ID NO: 4 - protein, 16 aa, Artificial Sequence
  Synthetic Construct
RSSQSLVHSNGNTYLH

SEQ ID NO: 5 - protein, 7 aa, Artificial Sequence
  Synthetic Construct
KVSNRFS

SEQ ID NO: 6 - protein, 9 aa, Artificial Sequence
  Synthetic Construct
SQSTHVPFT

SEQ ID NO: 7 - protein, 119 aa, Artificial Sequence
  Synthetic Construct
EVKLVESGGGLVQPGGSLRLSCATSGFTFTDYHLNWVRQPPGKALEWLALIRNKRYGYRTEYSASVKGRFTISRDNSQSILYLQMNTLRAEDSATYYCARDFYDPFAYWGQGTLVTVSA

SEQ ID NO: 8 - protein, 112 aa, Artificial Sequence
  Synthetic Construct
DVVMTQTPLSLPVSLGDQASISCRSSQSLVHSNGNTYLHWYLQRPGQSPKLLIYKVSNRFSGVPDRFSGSGSGTDFTLKISRVEAEDLGVYFCSQSTHVPFTFGSGTKLEIK

SEQ ID NO: 9 - protein, 15 aa, Artificial Sequence
  Synthetic Construct
GGGGSGGGGSGGGGS

SEQ ID NO: 10 - protein, 15 aa, Artificial Sequence
  Synthetic Construct
SSGGGGSGGGGSGGS

SEQ ID NO: 11 - protein, 18 aa, Artificial Sequence
  Synthetic Construct
GSTSGSGKPGSGEGSTKG

SEQ ID NO: 12 - protein, 284 aa, Artificial Sequence
  Synthetic Construct
MKLWLNWIFLVTLLNGIQCEVKLVESGGGLVQPGGSLRLSCATSGFTFTDYHLNWVRQPPGKALEWLALIRNKRYGYRTEYSASVKGRFTISRDNSQSILYLQMNTLRAEDSATYYCARDFYDPFAYWGQGTLVTVSAGGGGSGGGGSGGGGSMKLPVRLLVLMFWIPASSSDVVMTQTPLSLPVSLGDQASISCRSSQSLVHSNGNTYLHWYLQRPGQSPKLLIYKVSNRFSGVPDRFSGSGSGTDFTLKISRVEAEDLGVYFCSQSTHVPFTFGSGTKLEIK

SEQ ID NO: 13 - protein, 284 aa, Artificial Sequence
  Synthetic Construct
MKLPVRLLVLMFWIPASSSDVVMTQTPLSLPVSLGDQASISCRSSQSLVHSNGNTYLHWYLQRPGQSPKLLIYKVSNRFSGVPDRFSGSGSGTDFTLKISRVEAEDLGVYFCSQSTHVPFTFGSGTKLEIKGGGGSGGGGSGGGGSMKLWLNWIFLVTLLNGIQCEVKLVESGGGLVQPGGSLRLSCATSGFTFTDYHLNWVRQPPGKALEWLALIRNKRYGYRTEYSASVKGRFTISRDNSQSILYLQMNTLRAEDSATYYCARDFYDPFAYWGQGTLVTVSA

SEQ ID NO: 14 - protein, 13 aa, Artificial Sequence
  Synthetic Construct
CQTEPYYDLTSNA

SEQ ID NO: 15 - protein, 16 aa, Artificial Sequence
  Synthetic Construct
CALVHWPFGKAICRVV

SEQ ID NO: 16 - protein, 12 aa, Artificial Sequence
  Synthetic Construct
QTEPYYDLTSNA

SEQ ID NO: 17 - protein, 15 aa, Artificial Sequence
  Synthetic Construct
ALVHWPFGKAICRVV

SEQ ID NO: 18 - protein, 119 aa, Artificial Sequence
  Synthetic Construct
EVKLVESGGGLVQPGGSLRLSCATSGFTFTDYHMNWVRQPPGKALEWLALIRNKANGYRTEYSASVKGRFTISRDNSQNILYLQMNTLRAEDSATYYCARDFYDPFAYWGQGTLVTVSA

SEQ ID NO: 19 - protein, 112 aa, Artificial Sequence
  Synthetic Construct
DVVMTQTPLSLPVSLGDQASISCRSSQSLVHSNGNTYLHWYLQRPGQSPNLLIYKVSNRFSGVPDRFSGSGSGTDFTLKISRVEAEDLGLYFCSQSTRVPFTFGSGTKLEIK

SEQ ID NO: 20 - protein, 284 aa, Artificial Sequence
  Synthetic Construct
MKLWLNWIFPVTLLNGIQCEVKLVESGGGLVQPGGSLRLSCATSGFTFTDYHMNWVRQPPGKALEWLALIRNKANGYRTEYSASVKGRFTISRDNSQNILYLQMNTLRAEDSATYYCARDFYDPFAYWGQGTLVTVSAGGGGSGGGGSGGGGSMKLPVGLLVLMFWIPASSSDVVMTQTPLSLPVSLGDQASISCRSSQSLVHSNGNTYLHWYLQRPGQSPNLLIYKVSNRFSGVPDRFSGSGSGTDFTLKISRVEAEDLGLYFCSQSTRVPFTFGSGTKLEIK

SEQ ID NO: 21 - protein, 284 aa, Artificial Sequence
  Synthetic Construct
MKLPVGLLVLMFWIPASSSDVVMTQTPLSLPVSLGDQASISCRSSQSLVHSNGNTYLHWYLQRPGQSPNLLIYKVSNRFSGVPDRFSGSGSGTDFTLKISRVEAEDLGLYFCSQSTRVPFTFGSGTKLEIKGGGGSGGGGSGGGGSMKLWLNWIFPVTLLNGIQCEVKLVESGGGLVQPGGSLRLSCATSGFTFTDYHMNWVRQPPGKALEWLALIRNKANGYRTEYSASVKGRFTISRDNSQNILYLQMNTLRAEDSATYYCARDFYDPFAYWGQGTLVTVSA

SEQ ID NO: 22 - protein, 284 aa, Artificial Sequence
  Synthetic Construct
MKLWLNWIFLVTLLNGIQCEVKLVESGGGLVQPGGSLRLSCATSGFTFTDYHLNWVRQPPGKALEWLALIRNKRYGYRTEYSASVKGRFTISRDNSQSILYLQMNTLRAEDSATYYCARDFYDPFAYWGQGTLVTVSAGGGGSGGGGSGGGGSMKLPVGLLVLMFWIPASSSDVVMTQTPLSLPVSLGDQASISCRSSQSLVHSNGNTYLHWYLQRPGQSPNLLIYKVSNRFSGVPDRFSGSGSGTDFTLKISRVEAEDLGLYFCSQSTRVPFTFGSGTKLEIK

SEQ ID NO: 23 - protein, 284 aa, Artificial Sequence
  Synthetic Construct
MKLPVGLLVLMFWIPASSSDVVMTQTPLSLPVSLGDQASISCRSSQSLVHSNGNTYLHWYLQRPGQSPNLLIYKVSNRFSGVPDRFSGSGSGTDFTLKISRVEAEDLGLYFCSQSTRVPFTFGSGTKLEIKGGGGSGGGGSGGGGSMKLWLNWIFLVTLLNGIQCEVKLVESGGGLVQPGGSLRLSCATSGFTFTDYHLNWVRQPPGKALEWLALIRNKRYGYRTEYSASVKGRFTISRDNSQSILYLQMNTLRAEDSATYYCARDFYDPFAYWGQGTLVTVSA

SEQ ID NO: 24 - protein, 284 aa, Artificial Sequence
  Synthetic Construct
MKLWLNWIFPVTLLNGIQCEVKLVESGGGLVQPGGSLRLSCATSGFTFTDYHMNWVRQPPGKALEWLALIRNKANGYRTEYSASVKGRFTISRDNSQNILYLQMNTLRAEDSATYYCARDFYDPFAYWGQGTLVTVSAGGGGSGGGGSGGGGSMKLPVRLLVLMFWIPASSSDVVMTQTPLSLPVSLGDQASISCRSSQSLVHSNGNTYLHWYLQRPGQSPKLLIYKVSNRFSGVPDRFSGSGSGTDFTLKISRVEAEDLGVYFCSQSTHVPFTFGSGTKLEIK

SEQ ID NO: 25 - protein, 284 aa, Artificial Sequence
  Synthetic Construct
MKLPVRLLVLMFWIPASSSDVVMTQTPLSLPVSLGDQASISCRSSQSLVHSNGNTYLHWYLQRPGQSPKLLIYKVSNRFSGVPDRFSGSGSGTDFTLKISRVEAEDLGVYFCSQSTHVPFTFGSGTKLEIKGGGGSGGGGSGGGGSMKLWLNWIFPVTLLNGIQCEVKLVESGGGLVQPGGSLRLSCATSGFTFTDYHMNWVRQPPGKALEWLALIRNKANGYRTEYSASVKGRFTISRDNSQNILYLQMNTLRAEDSATYYCARDFYDPFAYWGQGTLVTVSA

SEQ ID NO: 26 - protein, 5 aa, Artificial Sequence
  Synthetic Construct
DYHMN

SEQ ID NO: 27 - protein, 19 aa, Artificial Sequence
  Synthetic Construct
LIRNKANGYRTEYSASVKG

SEQ ID NO: 28 - protein, 9 aa, Artificial Sequence
  Synthetic Construct
SQSTRVPFT

SEQ ID NO: 29 - protein, 19 aa, Artificial Sequence
  Synthetic Construct
MKLWLNWIFLVTLLNGIQC

SEQ ID NO: 30 - protein, 19 aa, Artificial Sequence
  Synthetic Construct
MKLPVGLLVLMFWIPASSS